European Patent Application EP 4 332 225 A1, published March 6, 2024. Title: Application of Artificially Synthesized CpG Single-stranded Deoxyoligonucleotide in Vaccines. Applicant: Parr Biotechnology (HeBei) Co., Ltd. Application PCT/CN2022/090392. The sequence listing filed with the application follows.

SEQUENCE LISTING (5 sequences)

SEQ ID NO: 1 - DNA, 23 bp, Artificial Sequence
  misc_feature: at least one nucleotide being a chemically modified nucleotide
tcgacgttcgtcgttcgtcgttc

SEQ ID NO: 2 - DNA, 24 bp, Artificial Sequence
  misc_feature: at least one nucleotide being a chemically modified nucleotide
tcgcgacgttcgccgacgttcgta

SEQ ID NO: 3 - DNA, 21 bp, Artificial Sequence
  misc_feature: at least one nucleotide being a chemically modified nucleotide
tcgtcgacgtcgttcgttctc

SEQ ID NO: 4 - DNA, 29 bp, Artificial Sequence
  misc_feature: at least one nucleotide being a chemically modified nucleotide
tcgcgaacgttcgccgcgtacgtacgcgg

SEQ ID NO: 5 - DNA, 22 bp, Artificial Sequence
  misc_feature: all nucleotides being phosphorothioated nucleotides
tgactgtgaacgttcgagatga